European Patent Application EP 4 218 798 A1, published August 2, 2023. Title: CANCER VACCINES TARGETING PRAME AND USES THEREOF. Applicant: INOVIO PHARMACEUTICALS, INC. Application EP. The sequence listing filed with the application follows.

SEQUENCE LISTING (2 sequences)

SEQ ID NO: 1 - DNA, 1584 bp, synthetic construct
  misc_feature 1..1584: note = Synthetic Consensus PRAME DNA Coding Sequence pGX1421
  source 1..1584: mol_type = other DNA
atggactggacatggattctgttcctggtcgctgctgctacacgggtgcattcagagagacgaagactgcggggctcaattcagagtaggtacatcagtatgtcagtctggacctcaccacggagactggtggaactggccgggcagagcctgctgaaggatgaggccctggctattgccgctctggaactgctgccccgagagctgttccctcccctgttcatggcagccttcgacggacgccacagccagactctgaaggctatggtccaggcatggccctttacctgcctgcctctgggcgtgctgatgaaggggcagcagctgcatctggagactttcaaagcagtgctggatggcctggacgtgctgctggcccaggaagtgaggcctaggcgctggaagctggaggtcctggatctgcgcaaaaacagccaccaggacttttggaccgtgtggtccgggaatcgggccagtctgtactcattcccagaacccgaggctgcacagccaatgcggaagaaaagaaaggtggatggactgtccaccgaagctgagcagccttttacaccaatcgaagtgctggtcgatctgtccctgaaagaaggcgcatgcgacgagctgttctcttatctgatggagaaggtcaaaagacagaagaacgtgctgcacctgtgctgtaagaaactgaaaatctttgctatgcccatgcaggacatcaagatgattctgaaaatggtccagctggattccattgaagacctggaggtcacttgtacctggaagctgccaacactggccaaattctctccctacctgggacagatgatcaatctgcgacggctgctgctgtctcacatccatgctagctcctctattagtcctgagaaggaggaagagtacattgcacagtttacttctcagttcctgagtctgcagtgcctgcaggccctgtatgtggatagcctgttctttctgagaggcaggctggaccagctgctgcgacacgtcatgaaccccctggaaacactgagtgtgactaattgtagactgtcagagggcgatgtgatgcatctgagccagtcccctaacgtgagccagctgtccgtcctgtctctgagtggcgtgatgctgacagacgtgagccctgaaccactgcaggccctgctggagcgagcatctgccactctgcaggacctggattttgacgagtgtgggatcatggacgatcagctgctggtgctgctgccttcactgagccactgctcccagctgaccacactgtctttctgtgggaacccaatctccatttctgtgctgcagaatctgctgcaccatctgattggactgagcaacctgacccatgtgctgtaccccgtccctctggaaagctatgaggatgtgcacggaacactgcatctgggcaggctggcctatctgcacgctcgcctgcgagaagtggtgtgcgagctgggcagaccctcaatggtgtggctgagcgccaatccatgtccccattgcggcgaccggacattctacgaccccgaacctattctgtgcccctgcttcatgcctaactgataa

SEQ ID NO: 2 - protein, 526 aa, synthetic construct
  REGION 1..526: note = Synthetic Consensus PRAME Protein Coding Sequence pGX1421
MDWTWILFLVAAATRVHSERRRLRGSIQSRYISMSVWTSPRRLVELAGQSLLKDEALAIAALELLPRELFPPLFMAAFDGRHSQTLKAMVQAWPFTCLPLGVLMKGQQLHLETFKAVLDGLDVLLAQEVRPRRWKLEVLDLRKNSHQDFWTVWSGNRASLYSFPEPEAAQPMRKKRKVDGLSTEAEQPFTPIEVLVDLSLKEGACDELFSYLMEKVKRQKNVLHLCCKKLKIFAMPMQDIKMILKMVQLDSIEDLEVTCTWKLPTLAKFSPYLGQMINLRRLLLSHIHASSSISPEKEEEYIAQFTSQFLSLQCLQALYVDSLFFLRGRLDQLLRHVMNPLETLSVTNCRLSEGDVMHLSQSPNVSQLSVLSLSGVMLTDVSPEPLQALLERASATLQDLDFDECGIMDDQLLVLLPSLSHCSQLTTLSFCGNPISISVLQNLLHHLIGLSNLTHVLYPVPLESYEDVHGTLHLGRLAYLHARLREVVCELGRPSMVWLSANPCPHCGDRTFYDPEPILCPCFMPN